European Patent Application EP 4 613 772 A2, published September 10, 2025. Title: Antigen-Binding Proteins That Antagonize Leptin Receptor. Applicant: Regeneron Pharmaceuticals, Inc. Application EP. The sequence listing filed with the application follows.

SEQUENCE LISTING (95 sequences)

SEQ ID NO: 1 - DNA, 378 bp, synthetic construct
  misc_feature 1..378: note = synthetic
  source 1..378: mol_type = other DNA
cagctgcagctgcaggagtcgggcccaggactggtgaagccttcggagaccctgtccctcacctgcactgtctctggtgcctctatcagcagtagtcgtttctacgggggctggatccgccagcccccagggaagggtctggagtggattggggatatctattatagtgggaatacctactacaacccgtccctccagagtcgagtcaccatatccgtagacacgtccaagaatcagttctccctgaagctgagctctgtgaccgccgcagacacggctgtgtattactgtgcgagacaccttatgattacgtttgggggacttatcgtcgagggttttgatatttggggccaagggacaatggtcaccgtctcttca

SEQ ID NO: 2 - protein, 126 aa, synthetic construct
  REGION 1..126: note = synthetic
QLQLQESGPGLVKPSETLSLTCTVSGASISSSRFYGGWIRQPPGKGLEWIGDIYYSGNTYYNPSLQSRVTISVDTSKNQFSLKLSSVTAADTAVYYCARHLMITFGGLIVEGFDIWGQGTMVTVSS

SEQ ID NO: 3 - DNA, 30 bp, synthetic construct
  misc_feature 1..30: note = synthetic
  source 1..30: mol_type = other DNA
ggtgcctctatcagcagtagtcgtttctac

SEQ ID NO: 4 - protein, 10 aa, synthetic construct
  REGION 1..10: note = synthetic
GASISSSRFY

SEQ ID NO: 5 - DNA, 21 bp, synthetic construct
  misc_feature 1..21: note = synthetic
  source 1..21: mol_type = other DNA
atctattatagtgggaatacc

SEQ ID NO: 6 - protein, 7 aa, synthetic construct
  REGION 1..7: note = synthetic
IYYSGNT

SEQ ID NO: 7 - DNA, 54 bp, synthetic construct
  misc_feature 1..54: note = synthetic
  source 1..54: mol_type = other DNA
gcgagacaccttatgattacgtttgggggacttatcgtcgagggttttgatatt

SEQ ID NO: 8 - protein, 18 aa, synthetic construct
  REGION 1..18: note = synthetic
ARHLMITFGGLIVEGFDI

SEQ ID NO: 9 - DNA, 324 bp, synthetic construct
  misc_feature 1..324: note = synthetic
  source 1..324: mol_type = other DNA
gacatccagatgacccagtctccatcctccctgtctgcatctgtaggagacagagtcaccatcacttgccgggcaagtcagagcattagcagctatttaaattggtatcagcagaaaccagggaaagcccctaagctcctgatctatgctgcatccagtttgcaaagtggggtcccgtcaaggttcagtggcagtggatctgggacagatttcactctcaccatcagcagtctgcaacctgaagattttgcaacttactactgtcaacagagttacagtacccctccgatcaccttcggccaagggacacgactggagattaaa

SEQ ID NO: 10 - protein, 108 aa, synthetic construct
  REGION 1..108: note = synthetic
DIQMTQSPSSLSASVGDRVTITCRASQSISSYLNWYQQKPGKAPKLLIYAASSLQSGVPSRFSGSGSGTDFTLTISSLQPEDFATYYCQQSYSTPPITFGQGTRLEIK

SEQ ID NO: 11 - DNA, 18 bp, synthetic construct
  misc_feature 1..18: note = synthetic
  source 1..18: mol_type = other DNA
cagagcattagcagctat

SEQ ID NO: 12 - protein, 6 aa, synthetic construct
  REGION 1..6: note = synthetic
QSISSY

SEQ ID NO: 13-14 - skipped (2 entries)

SEQ ID NO: 15 - DNA, 30 bp, synthetic construct
  misc_feature 1..30: note = synthetic
  source 1..30: mol_type = other DNA
caacagagttacagtacccctccgatcacc

SEQ ID NO: 16 - protein, 10 aa, synthetic construct
  REGION 1..10: note = synthetic
QQSYSTPPIT

SEQ ID NO: 17 - DNA, 366 bp, synthetic construct
  misc_feature 1..366: note = synthetic
  source 1..366: mol_type = other DNA
caggtgcagctggtggagtctgggggaggcgtggtccagcctgggaggtccctgagactctcctgtgcagcctctggattcactttcagtagctatggcatccactgggtccgccaggctccaggcaaggggctggagtgggtggcagttatatcatatgatggaaataataaatactatgcagactccgtgaagggccgattcaccatctccagagacaattccaagaacacgctgtatctgcaaatgaacagcctgagagctgaggacacggctgtatattactgtgcgaaagatctatttttggagtggttatttcacggtatgggcgtctggggccaagggaccacggtcaccgtctcctca

SEQ ID NO: 18 - protein, 122 aa, synthetic construct
  REGION 1..122: note = synthetic
QVQLVESGGGVVQPGRSLRLSCAASGFTFSSYGIHWVRQAPGKGLEWVAVISYDGNNKYYADSVKGRFTISRDNSKNTLYLQMNSLRAEDTAVYYCAKDLFLEWLFHGMGVWGQGTTVTVSS

SEQ ID NO: 19 - DNA, 24 bp, synthetic construct
  misc_feature 1..24: note = synthetic
  source 1..24: mol_type = other DNA
ggattcactttcagtagctatggc

SEQ ID NO: 20 - protein, 8 aa, synthetic construct
  REGION 1..8: note = synthetic
GFTFSSYG

SEQ ID NO: 21 - DNA, 24 bp, synthetic construct
  misc_feature 1..24: note = synthetic
  source 1..24: mol_type = other DNA
atatcatatgatggaaataataaa

SEQ ID NO: 22 - protein, 8 aa, synthetic construct
  REGION 1..8: note = synthetic
ISYDGNNK

SEQ ID NO: 23 - DNA, 45 bp, synthetic construct
  misc_feature 1..45: note = synthetic
  source 1..45: mol_type = other DNA
gcgaaagatctatttttggagtggttatttcacggtatgggcgtc

SEQ ID NO: 24 - protein, 15 aa, synthetic construct
  REGION 1..15: note = synthetic
AKDLFLEWLFHGMGV

SEQ ID NO: 25 - DNA, 372 bp, synthetic construct
  misc_feature 1..372: note = synthetic
  source 1..372: mol_type = other DNA
cagctgcagctgcaggagtcgggcccaggactagtgaagccttcggagaccctgtccctcacctgcattgtctctggtggcgacatcaccagtagtagttattactggaactggatccgccagcccccagggaaagggctggagtggattgggaatatctattatagtggaagcaccaactacaacccgtccctcaagagtcgagtcaccatatccatagacacgtccaagagccagttctccctgaagctgaggtctgtgaccgccgcagacacggctgtttattactgtgcgagattattacgatattttgactggtcaaaaggataccttgactactggggccagggaaccctggtcaccgtctcctca

SEQ ID NO: 26 - protein, 124 aa, synthetic construct
  REGION 1..124: note = synthetic
QLQLQESGPGLVKPSETLSLTCIVSGGDITSSSYYWNWIRQPPGKGLEWIGNIYYSGSTNYNPSLKSRVTISIDTSKSQFSLKLRSVTAADTAVYYCARLLRYFDWSKGYLDYWGQGTLVTVSS

SEQ ID NO: 27 - DNA, 30 bp, synthetic construct
  misc_feature 1..30: note = synthetic
  source 1..30: mol_type = other DNA
ggtggcgacatcaccagtagtagttattac

SEQ ID NO: 28 - protein, 10 aa, synthetic construct
  REGION 1..10: note = synthetic
GGDITSSSYY

SEQ ID NO: 29 - DNA, 21 bp, synthetic construct
  misc_feature 1..21: note = synthetic
  source 1..21: mol_type = other DNA
atctattatagtggaagcacc

SEQ ID NO: 30 - protein, 7 aa, synthetic construct
  REGION 1..7: note = synthetic
IYYSGST

SEQ ID NO: 31 - DNA, 48 bp, synthetic construct
  misc_feature 1..48: note = synthetic
  source 1..48: mol_type = other DNA
gcgagattattacgatattttgactggtcaaaaggataccttgactac

SEQ ID NO: 32 - protein, 16 aa, synthetic construct
  REGION 1..16: note = synthetic
ARLLRYFDWSKGYLDY

SEQ ID NO: 33 - DNA, 369 bp, synthetic construct
  misc_feature 1..369: note = synthetic
  source 1..369: mol_type = other DNA
caggtgcagctggtggagtctgggggaggcatggtcaagcctggagggtccctgagactctcctgtgcagcctctggattcaccttcagtgactactatatgagctggatccgccaggctccagggaagggtctggagtggatttcacacattagtattactggtagcaccatatactacgcagactctgtgaagggccgattcaccatctccagggacaacgccaagaattcactgtatttggaaatgaacagactgagagacgaggacacggccgtatattactgtacgagagatgagccggatattgtactagtaaggtacggtatggacgtctggggccaagggaccacggtcaccgtctcctca

SEQ ID NO: 34 - protein, 123 aa, synthetic construct
  REGION 1..123: note = synthetic
QVQLVESGGGMVKPGGSLRLSCAASGFTFSDYYMSWIRQAPGKGLEWISHISITGSTIYYADSVKGRFTISRDNAKNSLYLEMNRLRDEDTAVYYCTRDEPDIVLVRYGMDVWGQGTTVTVSS

SEQ ID NO: 35 - DNA, 24 bp, synthetic construct
  misc_feature 1..24: note = synthetic
  source 1..24: mol_type = other DNA
ggattcaccttcagtgactactat

SEQ ID NO: 36 - protein, 8 aa, synthetic construct
  REGION 1..8: note = synthetic
GFTFSDYY

SEQ ID NO: 37 - DNA, 24 bp, synthetic construct
  misc_feature 1..24: note = synthetic
  source 1..24: mol_type = other DNA
attagtattactggtagcaccata

SEQ ID NO: 38 - protein, 8 aa, synthetic construct
  REGION 1..8: note = synthetic
ISITGSTI

SEQ ID NO: 39 - DNA, 48 bp, synthetic construct
  misc_feature 1..48: note = synthetic
  source 1..48: mol_type = other DNA
acgagagatgagccggatattgtactagtaaggtacggtatggacgtc

SEQ ID NO: 40 - protein, 16 aa, synthetic construct
  REGION 1..16: note = synthetic
TRDEPDIVLVRYGMDV

SEQ ID NO: 41 - DNA, 351 bp, synthetic construct
  misc_feature 1..351: note = synthetic
  source 1..351: mol_type = other DNA
gaggtgcagctggtggagtctgggggaagtgtggtacggcctggggaatccctgagactctcctgtgcagcctctggattcacatttgatgattatggcatgagctgggtccgccaagctccagggaaggggctggagtgggtctctggtattagttggaatggtggcatcacagtttatgcagactctgtgaagggccgattcaccgtctccagagacaacgccaagaactccctgtatctgcaaatgaacagtctgagagccgaggacacggccctctatcactgtgcgagagcccgttatggtggcgccgactactggggccagggaaccctggtcaccgtctcctca

SEQ ID NO: 42 - protein, 117 aa, synthetic construct
  REGION 1..117: note = synthetic
EVQLVESGGSVVRPGESLRLSCAASGFTFDDYGMSWVRQAPGKGLEWVSGISWNGGITVYADSVKGRFTVSRDNAKNSLYLQMNSLRAEDTALYHCARARYGGADYWGQGTLVTVSS

SEQ ID NO: 43 - DNA, 24 bp, synthetic construct
  misc_feature 1..24: note = synthetic
  source 1..24: mol_type = other DNA
ggattcacatttgatgattatggc

SEQ ID NO: 44 - protein, 8 aa, synthetic construct
  REGION 1..8: note = synthetic
GFTFDDYG

SEQ ID NO: 45 - DNA, 24 bp, synthetic construct
  misc_feature 1..24: note = synthetic
  source 1..24: mol_type = other DNA
attagttggaatggtggcatcaca

SEQ ID NO: 46 - protein, 8 aa, synthetic construct
  REGION 1..8: note = synthetic
ISWNGGIT

SEQ ID NO: 47 - DNA, 30 bp, synthetic construct
  misc_feature 1..30: note = synthetic
  source 1..30: mol_type = other DNA
gcgagagcccgttatggtggcgccgactac

SEQ ID NO: 48 - protein, 10 aa, synthetic construct
  REGION 1..10: note = synthetic
ARARYGGADY

SEQ ID NO: 49 - DNA, 366 bp, synthetic construct
  misc_feature 1..366: note = synthetic
  source 1..366: mol_type = other DNA
gaggtgcagctggtggagtctgggggagacttggtacagcctgggcggtccctgagactctcctgtgcagcctctggattcacctttagcagttttgccatgagctgggtccgccaggctccagggaggggactggagtgggtctcaagtctcagtgatagtggtgataacacatactacgcagactccgtgaagggccggttcaccatctccagagacaattccaaaaatacgttgtatctgcaaatgaacaacctgagagccgaggacacggccgtttattactgtgcgaaagatctcttttcggggtggttattccatggttttgatgtctggggccaagggacaatggtcaccgtctcttca

SEQ ID NO: 50 - protein, 122 aa, synthetic construct
  REGION 1..122: note = synthetic
EVQLVESGGDLVQPGRSLRLSCAASGFTFSSFAMSWVRQAPGRGLEWVSSLSDSGDNTYYADSVKGRFTISRDNSKNTLYLQMNNLRAEDTAVYYCAKDLFSGWLFHGFDVWGQGTMVTVSS

SEQ ID NO: 51 - DNA, 24 bp, synthetic construct
  misc_feature 1..24: note = synthetic
  source 1..24: mol_type = other DNA
ggattcacctttagcagttttgcc

SEQ ID NO: 52 - protein, 8 aa, synthetic construct
  REGION 1..8: note = synthetic
GFTFSSFA

SEQ ID NO: 53 - DNA, 24 bp, synthetic construct
  misc_feature 1..24: note = synthetic
  source 1..24: mol_type = other DNA
ctcagtgatagtggtgataacaca

SEQ ID NO: 54 - protein, 8 aa, synthetic construct
  REGION 1..8: note = synthetic
LSDSGDNT

SEQ ID NO: 55 - DNA, 45 bp, synthetic construct
  misc_feature 1..45: note = synthetic
  source 1..45: mol_type = other DNA
gcgaaagatctcttttcggggtggttattccatggttttgatgtc

SEQ ID NO: 56 - protein, 15 aa, synthetic construct
  REGION 1..15: note = synthetic
AKDLFSGWLFHGFDV

SEQ ID NO: 57 - DNA, 351 bp, synthetic construct
  misc_feature 1..351: note = synthetic
  source 1..351: mol_type = other DNA
caggttcagctggtgcagtctggacctgaagtgaaaaaacctggggcctcagtgaaggtctcttgtaagggttctggttacaccttttcctggtatggaatcagctggatccgacaggcccctggacacggccttgaatggatgggatggatcagcgcttccagtggtaatacaagatttgcacagaaggtccagggcagactcaccatgaccacagacacatcgacgagtacagcctacatggagctgaggagcctgagatctgacgacacggccgtttattactgtgcgagaacggggactcggccctttgactattggggccagggaaccctggtcaccgtctcctca

SEQ ID NO: 58 - protein, 117 aa, synthetic construct
  REGION 1..117: note = synthetic
QVQLVQSGPEVKKPGASVKVSCKGSGYTFSWYGISWIRQAPGHGLEWMGWISASSGNTRFAQKVQGRLTMTTDTSTSTAYMELRSLRSDDTAVYYCARTGTRPFDYWGQGTLVTVSS

SEQ ID NO: 59 - DNA, 24 bp, synthetic construct
  misc_feature 1..24: note = synthetic
  source 1..24: mol_type = other DNA
ggttacaccttttcctggtatgga

SEQ ID NO: 60 - protein, 8 aa, synthetic construct
  REGION 1..8: note = synthetic
GYTFSWYG

SEQ ID NO: 61 - DNA, 24 bp, synthetic construct
  misc_feature 1..24: note = synthetic
  source 1..24: mol_type = other DNA
atcagcgcttccagtggtaataca

SEQ ID NO: 62 - protein, 8 aa, synthetic construct
  REGION 1..8: note = synthetic
ISASSGNT

SEQ ID NO: 63 - DNA, 30 bp, synthetic construct
  misc_feature 1..30: note = synthetic
  source 1..30: mol_type = other DNA
gcgagaacggggactcggccctttgactat

SEQ ID NO: 64 - protein, 10 aa, synthetic construct
  REGION 1..10: note = synthetic
ARTGTRPFDY

SEQ ID NO: 65 - DNA, 366 bp, synthetic construct
  misc_feature 1..366: note = synthetic
  source 1..366: mol_type = other DNA
gaggtgcagctggtggagtctgggggaggcttggtccagccgggggggtccctgagactctcctgtacagcctctggattcaccttcagtagctatggtctgcactgggtccgccaggctccagggaagggactggaatatgtttcaagtattaatcataatgggggtagtaaatattatgcagactctgtgaagggcagattcaccatctccagagacaattcgaagaacacgctgtttcttcaaatgggcagcctgaaaactgaggacatggctgtttattactgtgcgagagatctctttttggagtggttattccatggttttgatatctggggccaagggacaatggtcaccgtctcttca

SEQ ID NO: 66 - protein, 122 aa, synthetic construct
  REGION 1..122: note = synthetic
EVQLVESGGGLVQPGGSLRLSCTASGFTFSSYGLHWVRQAPGKGLEYVSSINHNGGSKYYADSVKGRFTISRDNSKNTLFLQMGSLKTEDMAVYYCARDLFLEWLFHGFDIWGQGTMVTVSS

SEQ ID NO: 67 - DNA, 24 bp, synthetic construct
  misc_feature 1..24: note = synthetic
  source 1..24: mol_type = other DNA
ggattcaccttcagtagctatggt

SEQ ID NO: 68 - protein, 8 aa, synthetic construct
  REGION 1..8: note = synthetic
GFTFSSYG

SEQ ID NO: 69 - DNA, 24 bp, synthetic construct
  misc_feature 1..24: note = synthetic
  source 1..24: mol_type = other DNA
attaatcataatgggggtagtaaa

SEQ ID NO: 70 - protein, 8 aa, synthetic construct
  REGION 1..8: note = synthetic
INHNGGSK

SEQ ID NO: 71 - DNA, 45 bp, synthetic construct
  misc_feature 1..45: note = synthetic
  source 1..45: mol_type = other DNA
gcgagagatctctttttggagtggttattccatggttttgatatc

SEQ ID NO: 72 - protein, 15 aa, synthetic construct
  REGION 1..15: note = synthetic
ARDLFLEWLFHGFDI

SEQ ID NO: 73 - DNA, 357 bp, synthetic construct
  misc_feature 1..357: note = synthetic
  source 1..357: mol_type = other DNA
caggtgcagctgcaggagtcgggcccaggactggtgaagccttcacagaccctgtccctcacctgttctgtctctggtggctccataaacactggttcttacttctggacttggatccgccagcacccaggggagggcctggagtggattgggtacatctattacaatggagacacctactacaatccgtccctcaagagtcgagttaccttatcactagacacgtctaagaaccagttctccctgaagctgaactctctgactgccggggacacggccgtttattactgtgcgagaagtgactggaactccctttttgaccactggggccaggggaccctggtcaccgtctcctca

SEQ ID NO: 74 - protein, 119 aa, synthetic construct
  REGION 1..119: note = synthetic
QVQLQESGPGLVKPSQTLSLTCSVSGGSINTGSYFWTWIRQHPGEGLEWIGYIYYNGDTYYNPSLKSRVTLSLDTSKNQFSLKLNSLTAGDTAVYYCARSDWNSLFDHWGQGTLVTVSS

SEQ ID NO: 75 - DNA, 30 bp, synthetic construct
  misc_feature 1..30: note = synthetic
  source 1..30: mol_type = other DNA
ggtggctccataaacactggttcttacttc

SEQ ID NO: 76 - protein, 10 aa, synthetic construct
  REGION 1..10: note = synthetic
GGSINTGSYF

SEQ ID NO: 77 - DNA, 21 bp, synthetic construct
  misc_feature 1..21: note = synthetic
  source 1..21: mol_type = other DNA
atctattacaatggagacacc

SEQ ID NO: 78 - protein, 7 aa, synthetic construct
  REGION 1..7: note = synthetic
IYYNGDT

SEQ ID NO: 79 - DNA, 33 bp, synthetic construct
  misc_feature 1..33: note = synthetic
  source 1..33: mol_type = other DNA
gcgagaagtgactggaactccctttttgaccac

SEQ ID NO: 80 - protein, 11 aa, synthetic construct
  REGION 1..11: note = synthetic
ARSDWNSLFDH

SEQ ID NO: 81 - DNA, 324 bp, synthetic construct
  misc_feature 1..324: note = synthetic
  source 1..324: mol_type = other DNA
gaaattgtgttgacgcagtctccaggcaccctgtctttgtctccaggggaaagagccaccctctcctgcagggccagtcagagtgttagcagcagctacttagcctggtaccagcagaaacctggccaggctcccaggctcctcatctatggtgcatccagcagggccactggcatcccagacaggttcagtggcagtgggtctgggacagacttcactctcaccatcagcagactggagcctgaagattttgcagtgtattactgtcagcagtatggtagctcaccttggacgttcggccaagggaccaaggtggaaatcaaa

SEQ ID NO: 82 - protein, 108 aa, synthetic construct
  REGION 1..108: note = synthetic
EIVLTQSPGTLSLSPGERATLSCRASQSVSSSYLAWYQQKPGQAPRLLIYGASSRATGIPDRFSGSGSGTDFTLTISRLEPEDFAVYYCQQYGSSPWTFGQGTKVEIK

SEQ ID NO: 83 - DNA, 21 bp, synthetic construct
  misc_feature 1..21: note = synthetic
  source 1..21: mol_type = other DNA
cagagtgttagcagcagctac

SEQ ID NO: 84 - protein, 7 aa, synthetic construct
  REGION 1..7: note = synthetic
QSVSSSY

SEQ ID NO: 85-86 - skipped (2 entries)

SEQ ID NO: 87 - DNA, 27 bp, synthetic construct
  misc_feature 1..27: note = synthetic
  source 1..27: mol_type = other DNA
cagcagtatggtagctcaccttggacg

SEQ ID NO: 88 - protein, 9 aa, synthetic construct
  REGION 1..9: note = synthetic
QQYGSSPWT

SEQ ID NO: 89 - protein, 1165 aa, synthetic construct
  REGION 1..1165: note = hLEPR P48357
MICQKFCVVLLHWEFIYVITAFNLSYPITPWRFKLSCMPPNSTYDYFLLPAGLSKNTSNSNGHYETAVEPKFNSSGTHFSNLSKTTFHCCFRSEQDRNCSLCADNIEGKTFVSTVNSLVFQQIDANWNIQCWLKGDLKLFICYVESLFKNLFRNYNYKVHLLYVLPEVLEDSPLVPQKGSFQMVHCNCSVHECCECLVPVPTAKLNDTLLMCLKITSGGVIFQSPLMSVQPINMVKPDPPLGLHMEITDDGNLKISWSSPPLVPFPLQYQVKYSENSTTVIREADKIVSATSLLVDSILPGSSYEVQVRGKRLDGPGIWSDWSTPRVFTTQDVIYFPPKILTSVGSNVSFHCIYKKENKIVPSKEIVWWMNLAEKIPQSQYDVVSDHVSKVTFFNLNETKPRGKFTYDAVYCCNEHECHHRYAELYVIDVNINISCETDGYLTKMTCRWSTSTIQSLAESTLQLRYHRSSLYCSDIPSIHPISEPKDCYLQSDGFYECIFQPIFLLSGYTMWIRINHSLGSLDSPPTCVLPDSVVKPLPPSSVKAEITINIGLLKISWEKPVFPENNLQFQIRYGLSGKEVQWKMYEVYDAKSKSVSLPVPDLCAVYAVQVRCKRLDGLGYWSNWSNPAYTVVMDIKVPMRGPEFWRIINGDTMKKEKNVTLLWKPLMKNDSLCSVQRYVINHHTSCNGTWSEDVGNHTKFTFLWTEQAHTVTVLAINSIGASVANFNLTFSWPMSKVNIVQSLSAYPLNSSCVIVSWILSPSDYKLMYFIIEWKNLNEDGEIKWLRISSSVKKYYIHDHFIPIEKYQFSLYPIFMEGVGKPKIINSFTQDDIEKHQSDAGLYVIVPVIISSSILLLGTLLISHQRMKKLFWEDVPNPKNCSWAQGLNFQKPETFEHLFIKHTASVTCGPLLLEPETISEDISVDTSWKNKDEMMPTTVVSLLSTTDLEKGSVCISDQFNSVNFSEAEGTEVTYEDESQRQPFVKYATLISNSKPSETGEEQGLINSSVTKCFSSKNSPLKDSFSNSSWEIEAQAFFILSDQHPNIISPHLTFSEGLDELLKLEGNFPEENNDKKSIYYLGVTSIKKRESGVLLTDKSRVSCPFPAPCLFTDIRVLQDSCSHFVENNINLGTSSKKTFASYMPQFQTCSTQTHKIMENKMCDLTV

SEQ ID NO: 90 - protein, 846 aa, synthetic construct
  REGION 1..846: note = hLEPR-mmh aa 1-818: F22-D839 of P48357 aa 819-846: myc-myc-hexahistidine tag
FNLSYPITPWRFKLSCMPPNSTYDYFLLPAGLSKNTSNSNGHYETAVEPKFNSSGTHFSNLSKTTFHCCFRSEQDRNCSLCADNIEGKTFVSTVNSLVFQQIDANWNIQCWLKGDLKLFICYVESLFKNLFRNYNYKVHLLYVLPEVLEDSPLVPQKGSFQMVHCNCSVHECCECLVPVPTAKLNDTLLMCLKITSGGVIFQSPLMSVQPINMVKPDPPLGLHMEITDDGNLKISWSSPPLVPFPLQYQVKYSENSTTVIREADKIVSATSLLVDSILPGSSYEVQVRGKRLDGPGIWSDWSTPRVFTTQDVIYFPPKILTSVGSNVSFHCIYKKENKIVPSKEIVWWMNLAEKIPQSQYDVVSDHVSKVTFFNLNETKPRGKFTYDAVYCCNEHECHHRYAELYVIDVNINISCETDGYLTKMTCRWSTSTIQSLAESTLQLRYHRSSLYCSDIPSIHPISEPKDCYLQSDGFYECIFQPIFLLSGYTMWIRINHSLGSLDSPPTCVLPDSVVKPLPPSSVKAEITINIGLLKISWEKPVFPENNLQFQIRYGLSGKEVQWKMYEVYDAKSKSVSLPVPDLCAVYAVQVRCKRLDGLGYWSNWSNPAYTVVMDIKVPMRGPEFWRIINGDTMKKEKNVTLLWKPLMKNDSLCSVQRYVINHHTSCNGTWSEDVGNHTKFTFLWTEQAHTVTVLAINSIGASVANFNLTFSWPMSKVNIVQSLSAYPLNSSCVIVSWILSPSDYKLMYFIIEWKNLNEDGEIKWLRISSSVKKYYIHDHFIPIEKYQFSLYPIFMEGVGKPKIINSFTQDDIEKHQSDEQKLISEEDLGGEQKLISEEDLHHHHHH

SEQ ID NO: 91 - protein, 1051 aa, synthetic construct
  REGION 1..1051: note = hLEPR-mFc aa 1-818: F22-D839 of P48357 aa 819-1051: mouse IgG2a (E98-K330 of P01863)
FNLSYPITPWRFKLSCMPPNSTYDYFLLPAGLSKNTSNSNGHYETAVEPKFNSSGTHFSNLSKTTFHCCFRSEQDRNCSLCADNIEGKTFVSTVNSLVFQQIDANWNIQCWLKGDLKLFICYVESLFKNLFRNYNYKVHLLYVLPEVLEDSPLVPQKGSFQMVHCNCSVHECCECLVPVPTAKLNDTLLMCLKITSGGVIFQSPLMSVQPINMVKPDPPLGLHMEITDDGNLKISWSSPPLVPFPLQYQVKYSENSTTVIREADKIVSATSLLVDSILPGSSYEVQVRGKRLDGPGIWSDWSTPRVFTTQDVIYFPPKILTSVGSNVSFHCIYKKENKIVPSKEIVWWMNLAEKIPQSQYDVVSDHVSKVTFFNLNETKPRGKFTYDAVYCCNEHECHHRYAELYVIDVNINISCETDGYLTKMTCRWSTSTIQSLAESTLQLRYHRSSLYCSDIPSIHPISEPKDCYLQSDGFYECIFQPIFLLSGYTMWIRINHSLGSLDSPPTCVLPDSVVKPLPPSSVKAEITINIGLLKISWEKPVFPENNLQFQIRYGLSGKEVQWKMYEVYDAKSKSVSLPVPDLCAVYAVQVRCKRLDGLGYWSNWSNPAYTVVMDIKVPMRGPEFWRIINGDTMKKEKNVTLLWKPLMKNDSLCSVQRYVINHHTSCNGTWSEDVGNHTKFTFLWTEQAHTVTVLAINSIGASVANFNLTFSWPMSKVNIVQSLSAYPLNSSCVIVSWILSPSDYKLMYFIIEWKNLNEDGEIKWLRISSSVKKYYIHDHFIPIEKYQFSLYPIFMEGVGKPKIINSFTQDDIEKHQSDEPRGPTIKPCPPCKCPAPNLLGGPSVFIFPPKIKDVLMISLSPIVTCVVVDVSEDDPDVQISWFVNNVEVHTAQTQTHREDYNSTLRVVSALPIQHQDWMSGKEFKCKVNNKDLPAPIERTISKPKGSVRAPQVYVLPPPEEEMTKKQVTLTCMVTDFMPEDIYVEWTNNGKTELNYKNTEPVLDSDGSYFMYSKLRVEKKNWVERNSYSCSVVHEGLHNHHTTKSFSRTPGK

SEQ ID NO: 92 - protein, 1045 aa, synthetic construct
  REGION 1..1045: note = hLEPR-hFc aa 1-818: F22-D839 of P48357 aa 819-1045: human IgG1 (D104-K330 of P01857)
FNLSYPITPWRFKLSCMPPNSTYDYFLLPAGLSKNTSNSNGHYETAVEPKFNSSGTHFSNLSKTTFHCCFRSEQDRNCSLCADNIEGKTFVSTVNSLVFQQIDANWNIQCWLKGDLKLFICYVESLFKNLFRNYNYKVHLLYVLPEVLEDSPLVPQKGSFQMVHCNCSVHECCECLVPVPTAKLNDTLLMCLKITSGGVIFQSPLMSVQPINMVKPDPPLGLHMEITDDGNLKISWSSPPLVPFPLQYQVKYSENSTTVIREADKIVSATSLLVDSILPGSSYEVQVRGKRLDGPGIWSDWSTPRVFTTQDVIYFPPKILTSVGSNVSFHCIYKKENKIVPSKEIVWWMNLAEKIPQSQYDVVSDHVSKVTFFNLNETKPRGKFTYDAVYCCNEHECHHRYAELYVIDVNINISCETDGYLTKMTCRWSTSTIQSLAESTLQLRYHRSSLYCSDIPSIHPISEPKDCYLQSDGFYECIFQPIFLLSGYTMWIRINHSLGSLDSPPTCVLPDSVVKPLPPSSVKAEITINIGLLKISWEKPVFPENNLQFQIRYGLSGKEVQWKMYEVYDAKSKSVSLPVPDLCAVYAVQVRCKRLDGLGYWSNWSNPAYTVVMDIKVPMRGPEFWRIINGDTMKKEKNVTLLWKPLMKNDSLCSVQRYVINHHTSCNGTWSEDVGNHTKFTFLWTEQAHTVTVLAINSIGASVANFNLTFSWPMSKVNIVQSLSAYPLNSSCVIVSWILSPSDYKLMYFIIEWKNLNEDGEIKWLRISSSVKKYYIHDHFIPIEKYQFSLYPIFMEGVGKPKIINSFTQDDIEKHQSDDKTHTCPPCPAPELLGGPSVFLFPPKPKDTLMISRTPEVTCVVVDVSHEDPEVKFNWYVDGVEVHNAKTKPREEQYNSTYRVVSVLTVLHQDWLNGKEYKCKVSNKALPAPIEKTISKAKGQPREPQVYTLPPSRDELTKNQVSLTCLVKGFYPSDIAVEWESNGQPENNYKTTPPVLDSDGSFFLYSKLTVDKSRWQQGNVFSCSVMHEALHNHYTQKSLSLSPGK

SEQ ID NO: 93 - protein, 844 aa, synthetic construct
  REGION 1..844: note = MfLEPR-mmh aa 1-816: Macaca fascicularis LEPR (F22-D837 of XP_005543194.1 with a T827A substitution) aa 817-844: myc-myc-hexahistidine tag
FNLSYPITPWRFKLSCMPPNSTYDYFLLPAGLSKNTSNLNGHYETAVEFNSSDTHFSNLSKTTFHCCFRSEQDRNCSLCADNIEGKTFVSTVNSSVFQQMGANWNIQCWLKGDLKLFICYVESLFKNPFKNYKHKVHLLYVLPEVLEDSPLVPQKGSFQMVHCNCSVHERCECLVPVPTAKLNDTLLMCLKITSGGVIFQSPLMSVQPINMVKPDPPLGLRMEITDDGNLKISWSSPPLVPFPLQYEVKYSENSTTVIREADKIVSATSLLVDGILPGSSYEVQVRGKRLDGPGIWSDWSTPHVFTTQDVIYFPPKILTSVGSNVSFHCIYKNENKIVSSKKIVWWMNLAEKIPQSQYDVVSDHVSKVTFFNLNETKPRGKFTYDAVYCCNEHECHHRYAELYVIDVNINISCETDGHLTKMTCRWSTNTIQSLAGSTLQLRYRRSSLYCFDIPSIHPISKPKDCYLQSDGFYECVFQPIFLLSGYTMWIRINHPLGSLDSPPTCVLPDSVVKPLPPSSVKAEIIKNIGLLKISWEKPVFPENNLQFQIRYGLSGKEIQWKMYDVYDAKSKSVSLPVPDFCAVYAVQVRCKRSDGLGLWSNWSNPAYTVVMDIKVPMRGPEFWRIINGDTMKKEKNVTLLWKPLMKNDSLCSVQRYVINHHTSCNGTWSEDVGNHTKFTFLWTEQAHTVTVLAINSIGASVANFNLTFSWPMSKVNIVQSLSAYPLNSSCVILSWILSPSDYKLMYFIIEWKNLNEDGEIKWLRISSSVKKYYIHDHFIPIEKYQFSLYPIFMEGVGKPKIINSFAQDNTEKHQNDEQKLISEEDLGGEQKLISEEDLHHHHHH

SEQ ID NO: 94 - protein, 846 aa, synthetic construct
  REGION 1..846: note = mLEPR-mmh aa 1-818: mouse LEPR (L22-G839 of NP_666258.2) aa 819-846: myc-myc-hexahistidine tag
LNLAYPISPWKFKLFCGPPNTTDDSFLSPAGAPNNASALKGASEAIVEAKFNSSGIYVPELSKTVFHCCFGNEQGQNCSALTDNTEGKTLASVVKASVFRQLGVNWDIECWMKGDLTLFICHMEPLPKNPFKNYDSKVHLLYDLPEVIDDSPLPPLKDSFQTVQCNCSLRGCECHVPVPRAKLNYALLMYLEITSAGVSFQSPLMSLQPMLVVKPDPPLGLHMEVTDDGNLKISWDSQTMAPFPLQYQVKYLENSTIVREAAEIVSATSLLVDSVLPGSSYEVQVRSKRLDGSGVWSDWSSPQVFTTQDVVYFPPKILTSVGSNASFHCIYKNENQIISSKQIVWWRNLAEKIPEIQYSIVSDRVSKVTFSNLKATRPRGKFTYDAVYCCNEQACHHRYAELYVIDVNINISCETDGYLTKMTCRWSPSTIQSLVGSTVQLRYHRRSLYCPDSPSIHPTSEPKNCVLQRDGFYECVFQPIFLLSGYTMWIRINHSLGSLDSPPTCVLPDSVVKPLPPSNVKAEITVNTGLLKVSWEKPVFPENNLQFQIRYGLSGKEIQWKTHEVFDAKSKSASLLVSDLCAVYVVQVRCRRLDGLGYWSNWSSPAYTLVMDVKVPMRGPEFWRKMDGDVTKKERNVTLLWKPLTKNDSLCSVRRYVVKHRTAHNGTWSEDVGNRTNLTFLWTEPAHTVTVLAVNSLGASLVNFNLTFSWPMSKVSAVESLSAYPLSSSCVILSWTLSPDDYSLLYLVIEWKILNEDDGMKWLRIPSNVKKFYIHDNFIPIEKYQFSLYPVFMEGVGKPKIINGFTKDAIDKQQNDAGEQKLISEEDLGGEQKLISEEDLHHHHHH

SEQ ID NO: 95 - protein, 846 aa, synthetic construct
  REGION 1..846: note = rLEPR-mmh aa 1-818: rat LEPR (L22-G839 of NP_036728.1) aa 819-846: myc-myc-hexahistidine tag
LNLAYPTSPWRFKLFCAPPSTTDDSFLSPAGVPNNTSSLKGASEALVEAKFNSTGIYVSELSKTIFHCCFGNEQGQNCSALTGNTEGKTLASVVKPLVFRQLGVNWDIECWMKGDLTLFICHMEPLLKNPFKNYDSKVHLLYDLPEVIDDLPLPPLKDSFQTVQCNCSVRECECHVPVPRAKVNYALLMYLEITSAGVSFQSPLMSLQPMLVVKPDPPLGLRMEVTDDGNLKISWDSQTKAPFPLQYQVKYLENSTIVREAAEIVSDTSLLVDSVLPGSSYEVQVRSKRLDGSGVWSDWSLPQLFTTQDVMYFPPKILTSVGSNASFCCIYKNENQTISSKQIVWWMNLAEKIPETQYNTVSDHISKVTFSNLKATRPRGKFTYDAVYCCNEQACHHRYAELYVIDVNINISCETDGYLTKMTCRWSPSTIQSLVGSTVQLRYHRRSLYCPDNPSIRPTSELKNCVLQTDGFYECVFQPIFLLSGYTMWIRINHSLGSLDSPPTCVLPDSVVKPLPPSNVKAEITINTGLLKVSWEKPVFPENNLQFQIRYGLNGKEIQWKTHEVFDAKSKSASLPVSDLCAVYVVQVRCRRLDGLGYWSNWSSPAYTLVMDVKVPMRGPEFWRIMDGDITKKERNVTLLWKPLMKNDSLCSVRRYVVKHRTAHNGTWSQDVGNQTNLTFLWAESAHTVTVLAINSIGASLVNFNLTFSWPMSKVNAVQSLSAYPLSSSCVILSWTLSPNDYSLLYLVIEWKNLNDDDGMKWLRIPSNVNKYYIHDNFIPIEKYQFSLYPVFMEGVGKPKIINGFTKDDIAKQQNDAGEQKLISEEDLGGEQKLISEEDLHHHHHH